European Patent Specification EP 3 574 020 B1, published May 15, 2024. Title: ANTIBODIES TO AMYLOID BETA. Applicant: THE UNIVERSITY OF BRITISH COLUMBIA PROMIS NEUROSCIENCES INC. The sequence listing filed with the application follows.

SEQUENCE LISTING (99 sequences)

SEQ ID NO: 1 - protein, 8 aa, Mus Musculus
GFTFSDYY

SEQ ID NO: 2 - protein, 8 aa, Mus Musculus
ISDGGSYT

SEQ ID NO: 3 - protein, 16 aa, Mus Musculus
ARDYYGSSSYTSGFAY

SEQ ID NO: 4 - protein, 12 aa, Mus Musculus
QSLLNSRTRKNY

SEQ ID NO: 5 - protein, 3 aa, Mus Musculus
WAS

SEQ ID NO: 6 - protein, 8 aa, Mus Musculus
KQSYNLYT

SEQ ID NO: 7 - protein, 4 aa, Homo Sapiens
HHQK

SEQ ID NO: 8 - DNA, 426 bp, Mus Musculus
atgaactttgggctcagcttgattttccttgtccttgttttaaaaggtgtccagtgtgaagtgcagctggtggagtctgggggaggcttagtgaagcctggagggtccctgaaactctcctgtgcagcctctggattcactttcagtgactattacatgtattgggttcgccagactccggaaaagaggctggagtgggtcgcaaccattagtgatggtggtagttacacctcctatccagacagtgtgaagggacgattcaccatctccagagacaatgccaagaacaacctgtacctgcaaatgagcagtctgaggtctgaggacacagccatgtattactgtgcaagagattactacggtagtagtagctacacctcgggctttgcttactggggccaagggactctggtcactgtctctgca

SEQ ID NO: 9 - protein, 142 aa, Mus Musculus
MNFGLSLIFLVLVLKGVQCEVQLVESGGGLVKPGGSLKLSCAASGFTFSDYYMYWVRQTPEKRLEWVATISDGGSYTSYPDSVKGRFTISRDNAKNNLYLQMSSLRSEDTAMYYCARDYYGSSSYTSGFAYWGQGTLVTVSA

SEQ ID NO: 10 - DNA, 396 bp, Mus Musculus
atggattcacaggcccaggttcttatattgctgctgctatgggtatctggtacctgtggggacattgtgatgtcacagtctccatcctccctggctgtgtcaacaggagagaaggtcactatgagctgcaaatccagtcagagtctgctcaacagtagaacccgaaagaactacttggcttggtaccagcagaaaccagggcagtctcctaaactgctgatctactgggcatccactagggaatctggggtccctgatcgcttcacaggcagtggatctgggacagatttcactctcaccatcagcagtgtgcaggctgaagacctggcagtttattactgcaagcaatcttataatctgtacacgttcggaggggggaccaagctggaaataaaa

SEQ ID NO: 11 - protein, 132 aa, Mus Musculus
MDSQAQVLILLLLWVSGTCGDIVMSQSPSSLAVSTGEKVTMSCKSSQSLLNSRTRKNYLAWYQQKPGQSPKLLIYWASTRESGVPDRFTGSGSGTDFTLTISSVQAEDLAVYYCKQSYNLYTFGGGTKLEIK

SEQ ID NO: 12 - protein, 7 aa, Artificial Sequence
  Artificial Construct
CGHHQKG

SEQ ID NO: 13 - DNA, 366 bp, Mus Musculus
caggtccaactgcagcagcctggggctgagcttgtgaagcctggggcttcagtgaagatgtcctgcaaggcttctggattcactttcagtgactattacataaactgggtgaagcagaggcctggacaaggccttgagtggattggagatattagtgatggtggtagttacacctacaatgctaagttcaagagcaaggccacactgactctggacacatcctccagcacagcctacatgcagctcagcagcctgacatctgaggactctgcggtctattactgtgcaagagattactacggtagtagtagctacacctcgggctttgcttactggggcgcaggcaccacggtcaccgtctcctca

SEQ ID NO: 14 - protein, 122 aa, Mus Musculus
QVQLQQPGAELVKPGASVKMSCKASGFTFSDYYINWVKQRPGQGLEWIGDISDGGSYTYNAKFKSKATLTLDTSSSTAYMQLSSLTSEDSAVYYCARDYYGSSSYTSGFAYWGAGTTVTVSS

SEQ ID NO: 15 - DNA, 366 bp, Artificial Sequence
  Synthetic Construct
caggtccaactggtgcagtctggggctgagcttaagaagcctggggcttcagtgaagatgtcctgcaaggcttctggattcactttcagtgactattacataaactgggtgaagcagaggcctggacaaggccttgagtggattggagatattagtgatggtggtagttacacctacaatgctaagttcaagagcagagccacactgactctggacacatccataagcacagcctacatgcagctcagcagcctgacatctgaggactctgcggtctattactgtgcaagagattactacggtagtagtagctacacctcgggctttgcttactggggccaaggcaccacggtcaccgtctcctca

SEQ ID NO: 16 - protein, 122 aa, Artificial Sequence
  Synthetic Construct
QVQLVQSGAELKKPGASVKMSCKASGFTFSDYYINWVKQRPGQGLEWIGDISDGGSYTYNAKFKSRATLTLDTSISTAYMQLSSLTSEDSAVYYCARDYYGSSSYTSGFAYWGQGTTVTVSS

SEQ ID NO: 17 - DNA, 366 bp, Artificial Sequence
  Synthetic Construct
caggtccaactggtgcagtctggggctgaggtgaagaagcctggggcttcagtgaagatgtcctgcaaggcttctggattcactttcagtgactattacataaactgggtgaagcagaggcctggacaaggccttgagtggattggagatattagtgatggtggtagttacacctacaatgctaagttcaagagcagagccacactgactctggacacatccataagcacagcctacatggagctcagcagcctgagatctgaggacacggcggtctattactgtgcaagagattactacggtagtagtagctacacctcgggctttgcttactggggccaaggcaccacggtcaccgtctcctca

SEQ ID NO: 18 - protein, 122 aa, Artificial Sequence
  Synthetic Construct
QVQLVQSGAEVKKPGASVKMSCKASGFTFSDYYINWVKQRPGQGLEWIGDISDGGSYTYNAKFKSRATLTLDTSISTAYMELSSLRSEDTAVYYCARDYYGSSSYTSGFAYWGQGTTVTVSS

SEQ ID NO: 19 - DNA, 366 bp, Artificial Sequence
  Synthetic Construct
caggtccaactggtgcagtctggggctgaggtgaagaagcctggggcttcagtgaaggtgtcctgcaaggcttctggattcactttcagtgactattacataaactgggtgcgacagaggcctggacaaggccttgagtggattggagatattagtgatggtggtagttacacctacaatgctaagttcaagagcagagccacactgactctggacacatccataagcacagcctacatggagctcagcagcctgagatctgaggacacggcggtctattactgtgcaagagattactacggtagtagtagctacacctcgggctttgcttactggggccaaggcaccacggtcaccgtctcctca

SEQ ID NO: 20 - protein, 122 aa, Artificial Sequence
  Synthetic Construct
QVQLVQSGAEVKKPGASVKVSCKASGFTFSDYYINWVRQRPGQGLEWIGDISDGGSYTYNAKFKSRATLTLDTSISTAYMELSSLRSEDTAVYYCARDYYGSSSYTSGFAYWGQGTTVTVSS

SEQ ID NO: 21 - DNA, 366 bp, Artificial Sequence
  Synthetic Construct
caggtccaactggtgcagtctggggctgaggtgaagaagcctggggcttcagtgaaggtgtcctgcaaggcttctggattcactttcagtgactattacataaactgggtgcgacagaggcctggacaaggccttgagtggattggagatattagtgatggtggtagttacacctacaatgctaagttcaagagcagagtcacactgactctggacacatccataagcacagcctacatggagctcagcagcctgagatctgaggacacggcggtctattactgtgcaagagattactacggtagtagtagctacacctcgggctttgcttactggggccaaggcaccacggtcaccgtctcctca

SEQ ID NO: 22 - protein, 122 aa, Artificial Sequence
  Synthetic Construct
QVQLVQSGAEVKKPGASVKVSCKASGFTFSDYYINWVRQRPGQGLEWIGDISDGGSYTYNAKFKSRVTLTLDTSISTAYMELSSLRSEDTAVYYCARDYYGSSSYTSGFAYWGQGTTVTVSS

SEQ ID NO: 23 - DNA, 366 bp, Artificial Sequence
  Synthetic Construct
caggtccaactggtgcagtctggggctgaggtgaagaagcctggggcttcagtgaaggtgtcctgcaaggcttctggattcactttcagtgactattacataaactgggtgcgacagaggcctggacaaggccttgagtggatgggagatattagtgatggtggtagttacacctacaatgctaagttcaagagcagagtcacactgactagggacacatccataagcacagcctacatggagctcagcagcctgagatctgaggacacggcggtctattactgtgcaagagattactacggtagtagtagctacacctcgggctttgcttactggggccaaggcaccacggtcaccgtctcctca

SEQ ID NO: 24 - protein, 122 aa, Artificial Sequence
  Synthetic Construct
QVQLVQSGAEVKKPGASVKVSCKASGFTFSDYYINWVRQRPGQGLEWMGDISDGGSYTYNAKFKSRVTLTRDTSISTAYMELSSLRSEDTAVYYCARDYYGSSSYTSGFAYWGQGTTVTVSS

SEQ ID NO: 25 - DNA, 366 bp, Artificial Sequence
  Synthetic Construct
caggtccaactggtgcagtctggggctgaggtgaagaagcctggggcttcagtgaaggtgtcctgcaaggcttctggattcactttcagtgactattacataaactgggtgcgacagaggcctggacaaggccttgagtggatgggagatattagtgatggtggtagttacacctacaatgctaagttccagggcagagtcacaatgactagggacacatccataagcacagcctacatggagctcagcagcctgagatctgaggacacggcggtctattactgtgcaagagattactacggtagtagtagctacacctcgggctttgcttactggggccaaggcaccacggtcaccgtctcctca

SEQ ID NO: 26 - protein, 122 aa, Artificial Sequence
  Synthetic Construct
QVQLVQSGAEVKKPGASVKVSCKASGFTFSDYYINWVRQRPGQGLEWMGDISDGGSYTYNAKFQGRVTMTRDTSISTAYMELSSLRSEDTAVYYCARDYYGSSSYTSGFAYWGQGTTVTVSS

SEQ ID NO: 27 - DNA, 336 bp, Mus Musculus
gatgttttgatgacccaaactccactctccctgcctgtcagtcttggagatcaagcctccatctcttgcagatctagtcagagtctgctcaacagtagaacccgaaagaactacttagaatggtacctgcagaaaccaggccagtctccaaagctcctgatctactgggcatccaaccgattttctggggtcccagacaggttcagtggcagtggatcagggacagatttcacactcaagatcagcagagtggaggctgaggatctgggagtttattactgcaagcaatcttataatctgtacacgtttggcagcgggaccaagctggagatcaaa

SEQ ID NO: 28 - protein, 112 aa, Mus Musculus
DVLMTQTPLSLPVSLGDQASISCRSSQSLLNSRTRKNYLEWYLQKPGQSPKLLIYWASNRFSGVPDRFSGSGSGTDFTLKISRVEAEDLGVYYCKQSYNLYTFGSGTKLEIK

SEQ ID NO: 29 - DNA, 336 bp, Artificial Sequence
  Synthetic Construct
gatgttttgatgacccaatctccactctccctgcctgtcacccttggacagccggcctccatctcttgcagatctagtcagagtctgctcaacagtagaacccgaaagaactacttagaatggtttcagcagaaaccaggccagtctccaaggcgcctgatctactgggcatccaaccgattttctggggtcccagacaggttcagtggcagtggatcagggacagatttcacactcaagatcagcagagtggaggctgaggatgttggagtttattactgcaagcaatcttataatctgtacacgtttggccaagggaccaagctggagatcaaa

SEQ ID NO: 30 - protein, 112 aa, Artificial Sequence
  Synthetic Construct
DVLMTQSPLSLPVTLGQPASISCRSSQSLLNSRTRKNYLEWFQQKPGQSPRRLIYWASNRFSGVPDRFSGSGSGTDFTLKISRVEAEDVGVYYCKQSYNLYTFGQGTKLEIK

SEQ ID NO: 31 - DNA, 336 bp, Artificial Sequence
  Synthetic Construct
gatgttgtgatgacccaatctccactctccctgcctgtcacccttggacagccggcctccatctcttgcagatctagtcagagtctgctcaacagtagaacccgaaagaactacttagaatggtttcagcagaaaccaggccagtctccaaggcgcctgatctactgggcatccaaccgattttctggggtcccagacaggttcagtggcagtggatcagggacagatttcacactcaagatcagcagagtggaggctgaggatgttggagtttattactgcaagcaatcttataatctgtacacgtttggccaagggaccaagctggagatcaaa

SEQ ID NO: 32 - protein, 112 aa, Artificial Sequence
  Synthetic Construct
DVVMTQSPLSLPVTLGQPASISCRSSQSLLNSRTRKNYLEWFQQKPGQSPRRLIYWASNRFSGVPDRFSGSGSGTDFTLKISRVEAEDVGVYYCKQSYNLYTFGQGTKLEIK

SEQ ID NO: 33 - DNA, 336 bp, Artificial Sequence
  Synthetic Construct
gatgttgtgatgacccaatctccactctccctgcctgtcacccttggacagccggcctccatctcttgcagatctagtcagagtctgctcaacagtagaacccgaaagaactacttagaatggtttcagcagaggccaggccagtctccaaggcgcctgatctactgggcatccaaccgattttctggggtcccagacaggttcagtggcagtggatcagggacagatttcacactcaagatcagcagagtggaggctgaggatgttggagtttattactgcaagcaatcttataatctgtacacgtttggccaagggaccaagctggagatcaaa

SEQ ID NO: 34 - protein, 112 aa, Artificial Sequence
  Synthetic Construct
DVVMTQSPLSLPVTLGQPASISCRSSQSLLNSRTRKNYLEWFQQRPGQSPRRLIYWASNRFSGVPDRFSGSGSGTDFTLKISRVEAEDVGVYYCKQSYNLYTFGQGTKLEIK

SEQ ID NO: 35 - DNA, 336 bp, Artificial Sequence
  Synthetic Construct
gatgttctgatgacccaatctccactctccctgcctgtcacccttggacagccggcctccatctcttgcagatctagtcagagtctgctcaacagtagaacccgaaagaactacttagaatggtacctgcagaggccaggccagtctccaaagctgctgatctactgggcatccaaccgattttctggggtcccagacaggttcagtggcagtggatcagggacagatttcacactcaagatcagcagagtggaggctgaggatgttggagtttattactgcaagcaatcttataatctgtacacgtttggccaagggaccaagctggagatcaaa

SEQ ID NO: 36 - protein, 112 aa, Artificial Sequence
  Synthetic Construct
DVLMTQSPLSLPVTLGQPASISCRSSQSLLNSRTRKNYLEWYLQRPGQSPKLLIYWASNRFSGVPDRFSGSGSGTDFTLKISRVEAEDVGVYYCKQSYNLYTFGQGTKLEIK

SEQ ID NO: 37 - DNA, 336 bp, Artificial Sequence
  Synthetic Construct
gatgttctgatgacccaatctccactctccctgcctgtcacccttggacagccggcctccatctcttgcagatctagtcagagtctgctcaacagtagaacccgaaagaactacttagaatggtaccagcagaggccaggccagtctccaaggctgctgatctactgggcatccaaccgattttctggggtcccagacaggttcagtggcagtggatcagggacagatttcacactcaagatcagcagagtggaggctgaggatgttggagtttattactgcaagcaatcttataatctgtacacgtttggccaagggaccaagctggagatcaaa

SEQ ID NO: 38 - protein, 112 aa, Artificial Sequence
  Synthetic Construct
DVLMTQSPLSLPVTLGQPASISCRSSQSLLNSRTRKNYLEWYQQRPGQSPRLLIYWASNRFSGVPDRFSGSGSGTDFTLKISRVEAEDVGVYYCKQSYNLYTFGQGTKLEIK

SEQ ID NO: 39 - DNA, 336 bp, Artificial Sequence
  Synthetic Construct
gatgttgtgatgacccaatctccactctccctgcctgtcacccttggacagccggcctccatctcttgcagatctagtcagagtctgctcaacagtagaacccgaaagaactacttagaatggtaccagcagaggccaggccagtctccaaggctgctgatctactgggcatccaaccgattttctggggtcccagacaggttcagtggcagtggatcagggacagatttcacactcaagatcagcagagtggaggctgaggatgttggagtttattactgcaagcaatcttataatctgtacacgtttggccaagggaccaagctggagatcaaa

SEQ ID NO: 40 - protein, 112 aa, Artificial Sequence
  Synthetic Construct
DVVMTQSPLSLPVTLGQPASISCRSSQSLLNSRTRKNYLEWYQQRPGQSPRLLIYWASNRFSGVPDRFSGSGSGTDFTLKISRVEAEDVGVYYCKQSYNLYTFGQGTKLEIK

SEQ ID NO: 41 - DNA, 360 bp, Mus Musculus
caggtccaactgcagcagcctggggctgagcttgtgaagcctggggcttcagtgaagatgtcctgcaaggcttctggctacagcttcaccagctactggataaactgggtgaagcagaggcctggacaaggccttgagtggattggagatgtgcatcctggtagaggcgtgtccacatacaatgctaagttcaagagcaaggccacactgactctggacacatcctccagcacagcctacatgcagctcagcagcctgacatctgaggactctgcggtctattactgtagcagatcccatggtaacacctactggttttttgacgtctggggcgcaggcaccacggtcaccgtctcctca

SEQ ID NO: 42 - protein, 120 aa, Mus Musculus
QVQLQQPGAELVKPGASVKMSCKASGYSFTSYWINWVKQRPGQGLEWIGDVHPGRGVSTYNAKFKSKATLTLDTSSSTAYMQLSSLTSEDSAVYYCSRSHGNTYWFFDVWGAGTTVTVSS

SEQ ID NO: 43 - DNA, 360 bp, Artificial Sequence
  Synthetic Construct
caggtccaactggtgcagtctggggctgagcttaagaagcctggggcttcagtgaagatgtcctgcaaggcttctggctacagcttcaccagctactggataaactgggtgaagcagaggcctggacaaggccttgagtggattggagatgtgcatcctggtagaggcgtgtccacatacaatgctaagttcaagagcagagccacactgactctggacacatccataagcacagcctacatgcagctcagcagcctgacatctgaggactctgcggtctattactgtagcagatcccatggtaacacctactggttttttgacgtctggggccaaggcaccacggtcaccgtctcctca

SEQ ID NO: 44 - protein, 120 aa, Artificial Sequence
  Synthetic Construct
QVQLVQSGAELKKPGASVKMSCKASGYSFTSYWINWVKQRPGQGLEWIGDVHPGRGVSTYNAKFKSRATLTLDTSISTAYMQLSSLTSEDSAVYYCSRSHGNTYWFFDVWGQGTTVTVSS

SEQ ID NO: 45 - DNA, 360 bp, Artificial Sequence
  Synthetic Construct
caggtccaactggtgcagtctggggctgaggtgaagaagcctggggcttcagtgaagatgtcctgcaaggcttctggctacagcttcaccagctactggataaactgggtgaagcagaggcctggacaaggccttgagtggattggagatgtgcatcctggtagaggcgtgtccacatacaatgctaagttcaagagcagagccacactgactctggacacatccataagcacagcctacatggagctcagcagcctgagatctgaggacacggcggtctattactgtagcagatcccatggtaacacctactggttttttgacgtctggggccaaggcaccacggtcaccgtctcctca

SEQ ID NO: 46 - protein, 120 aa, Artificial Sequence
  Synthetic Construct
QVQLVQSGAEVKKPGASVKMSCKASGYSFTSYWINWVKQRPGQGLEWIGDVHPGRGVSTYNAKFKSRATLTLDTSISTAYMELSSLRSEDTAVYYCSRSHGNTYWFFDVWGQGTTVTVSS

SEQ ID NO: 47 - DNA, 360 bp, Artificial Sequence
  Synthetic Construct
caggtccaactggtgcagtctggggctgaggtgaagaagcctggggcttcagtgaaggtgtcctgcaaggcttctggctacagcttcaccagctactggataaactgggtgcgacagaggcctggacaaggccttgagtggattggagatgtgcatcctggtagaggcgtgtccacatacaatgctaagttcaagagcagagccacactgactctggacacatccataagcacagcctacatggagctcagcagcctgagatctgaggacacggcggtctattactgtagcagatcccatggtaacacctactggttttttgacgtctggggccaaggcaccacggtcaccgtctcctca

SEQ ID NO: 48 - protein, 120 aa, Artificial Sequence
  Synthetic Construct
QVQLVQSGAEVKKPGASVKVSCKASGYSFTSYWINWVRQRPGQGLEWIGDVHPGRGVSTYNAKFKSRATLTLDTSISTAYMELSSLRSEDTAVYYCSRSHGNTYWFFDVWGQGTTVTVSS

SEQ ID NO: 49 - DNA, 360 bp, Artificial Sequence
  Synthetic Construct
caggtccaactggtgcagtctggggctgaggtgaagaagcctggggcttcagtgaaggtgtcctgcaaggcttctggctacagcttcaccagctactggataaactgggtgcgacagaggcctggacaaggccttgagtggattggagatgtgcatcctggtagaggcgtgtccacatacaatgctaagttcaagagcagagtcacactgactctggacacatccataagcacagcctacatggagctcagcagcctgagatctgaggacacggcggtctattactgtagcagatcccatggtaacacctactggttttttgacgtctggggccaaggcaccacggtcaccgtctcctca

SEQ ID NO: 50 - protein, 120 aa, Artificial Sequence
  Synthetic Construct
QVQLVQSGAEVKKPGASVKVSCKASGYSFTSYWINWVRQRPGQGLEWIGDVHPGRGVSTYNAKFKSRVTLTLDTSISTAYMELSSLRSEDTAVYYCSRSHGNTYWFFDVWGQGTTVTVSS

SEQ ID NO: 51 - DNA, 360 bp, Artificial Sequence
  Synthetic Construct
caggtccaactggtgcagtctggggctgaggtgaagaagcctggggcttcagtgaaggtgtcctgcaaggcttctggctacagcttcaccagctactggataaactgggtgcgacagaggcctggacaaggccttgagtggatgggagatgtgcatcctggtagaggcgtgtccacatacaatgctaagttcaagagcagagtcacactgactagggacacatccataagcacagcctacatggagctcagcagcctgagatctgaggacacggcggtctattactgtagcagatcccatggtaacacctactggttttttgacgtctggggccaaggcaccacggtcaccgtctcctca

SEQ ID NO: 52 - protein, 120 aa, Artificial Sequence
  Synthetic Construct
QVQLVQSGAEVKKPGASVKVSCKASGYSFTSYWINWVRQRPGQGLEWMGDVHPGRGVSTYNAKFKSRVTLTRDTSISTAYMELSSLRSEDTAVYYCSRSHGNTYWFFDVWGQGTTVTVSS

SEQ ID NO: 53 - DNA, 360 bp, Artificial Sequence
  Synthetic Construct
caggtccaactggtgcagtctggggctgaggtgaagaagcctggggcttcagtgaaggtgtcctgcaaggcttctggctacagcttcaccagctactggataaactgggtgcgacagaggcctggacaaggccttgagtggatgggagatgtgcatcctggtagaggcgtgtccacatacaatgctaagttccagggcagagtcacaatgactagggacacatccataagcacagcctacatggagctcagcagcctgagatctgaggacacggcggtctattactgtagcagatcccatggtaacacctactggttttttgacgtctggggccaaggcaccacggtcaccgtctcctca

SEQ ID NO: 54 - protein, 120 aa, Artificial Sequence
  Synthetic Construct
QVQLVQSGAEVKKPGASVKVSCKASGYSFTSYWINWVRQRPGQGLEWMGDVHPGRGVSTYNAKFQGRVTMTRDTSISTAYMELSSLRSEDTAVYYCSRSHGNTYWFFDVWGQGTTVTVSS

SEQ ID NO: 55 - DNA, 336 bp, Mus Musculus
gatgttttgatgacccaaactccactctccctgcctgtcagtcttggagatcaagcctccatctcttgcagatctagtcagagcattgtacatagtaatggaaacacctatttagaatggtacctgcagaaaccaggccagtctccaaagctcctgatctacaaagtttccaaccgattttctggggtcccagacaggttcagtggcagtggatcagggacagatttcacactcaagatcagcagagtggaggctgaggatctgggagtttattactgctttcaaggttcacatgttcctttcacttttggcagcgggaccaagctggagatcaaa

SEQ ID NO: 56 - protein, 112 aa, Mus Musculus
DVLMTQTPLSLPVSLGDQASISCRSSQSIVHSNGNTYLEWYLQKPGQSPKLLIYKVSNRFSGVPDRFSGSGSGTDFTLKISRVEAEDLGVYYCFQGSHVPFTFGSGTKLEIK

SEQ ID NO: 57 - DNA, 336 bp, Artificial Sequence
  Synthetic Construct
gatgttttgatgacccaatctccactctccctgcctgtcacccttggacagccggcctccatctcttgcagatctagtcagagcattgtacatagtaatggaaacacctatttagaatggtttcagcagaaaccaggccagtctccaaggcgcctgatctacaaagtttccaaccgattttctggggtcccagacaggttcagtggcagtggatcagggacagatttcacactcaagatcagcagagtggaggctgaggatgttggagtttattactgctttcaaggttcacatgttcctttcacttttggccaagggaccaagctggagatcaaa

SEQ ID NO: 58 - protein, 112 aa, Artificial Sequence
  Synthetic Construct
DVLMTQSPLSLPVTLGQPASISCRSSQSIVHSNGNTYLEWFQQKPGQSPRRLIYKVSNRFSGVPDRFSGSGSGTDFTLKISRVEAEDVGVYYCFQGSHVPFTFGQGTKLEIK

SEQ ID NO: 59 - DNA, 336 bp, Artificial Sequence
  Synthetic Construct
gatgttgtgatgacccaatctccactctccctgcctgtcacccttggacagccggcctccatctcttgcagatctagtcagagcattgtacatagtaatggaaacacctatttagaatggtttcagcagaaaccaggccagtctccaaggcgcctgatctacaaagtttccaaccgattttctggggtcccagacaggttcagtggcagtggatcagggacagatttcacactcaagatcagcagagtggaggctgaggatgttggagtttattactgctttcaaggttcacatgttcctttcacttttggccaagggaccaagctggagatcaaa

SEQ ID NO: 60 - protein, 112 aa, Artificial Sequence
  Synthetic Construct
DVVMTQSPLSLPVTLGQPASISCRSSQSIVHSNGNTYLEWFQQKPGQSPRRLIYKVSNRFSGVPDRFSGSGSGTDFTLKISRVEAEDVGVYYCFQGSHVPFTFGQGTKLEIK

SEQ ID NO: 61 - DNA, 336 bp, Artificial Sequence
  Synthetic Construct
gatgttgtgatgacccaatctccactctccctgcctgtcacccttggacagccggcctccatctcttgcagatctagtcagagcattgtacatagtaatggaaacacctatttagaatggtttcagcagaggccaggccagtctccaaggcgcctgatctacaaagtttccaaccgattttctggggtcccagacaggttcagtggcagtggatcagggacagatttcacactcaagatcagcagagtggaggctgaggatgttggagtttattactgctttcaaggttcacatgttcctttcacttttggccaagggaccaagctggagatcaaa

SEQ ID NO: 62 - protein, 112 aa, Artificial Sequence
  Synthetic Construct
DVVMTQSPLSLPVTLGQPASISCRSSQSIVHSNGNTYLEWFQQRPGQSPRRLIYKVSNRFSGVPDRFSGSGSGTDFTLKISRVEAEDVGVYYCFQGSHVPFTFGQGTKLEIK

SEQ ID NO: 63 - DNA, 336 bp, Artificial Sequence
  Synthetic Construct
gatgttctgatgacccaatctccactctccctgcctgtcacccttggacagccggcctccatctcttgcagatctagtcagagcattgtacatagtaatggaaacacctatttagaatggtacctgcagaggccaggccagtctccaaagctgctgatctacaaagtttccaaccgattttctggggtcccagacaggttcagtggcagtggatcagggacagatttcacactcaagatcagcagagtggaggctgaggatgttggagtttattactgctttcaaggttcacatgttcctttcacttttggccaagggaccaagctggagatcaaa

SEQ ID NO: 64 - protein, 112 aa, Artificial Sequence
  Synthetic Construct
DVLMTQSPLSLPVTLGQPASISCRSSQSIVHSNGNTYLEWYLQRPGQSPKLLIYKVSNRFSGVPDRFSGSGSGTDFTLKISRVEAEDVGVYYCFQGSHVPFTFGQGTKLEIK

SEQ ID NO: 65 - DNA, 336 bp, Artificial Sequence
  Synthetic Construct
gatgttctgatgacccaatctccactctccctgcctgtcacccttggacagccggcctccatctcttgcagatctagtcagagcattgtacatagtaatggaaacacctatttagaatggtaccagcagaggccaggccagtctccaaggctgctgatctacaaagtttccaaccgattttctggggtcccagacaggttcagtggcagtggatcagggacagatttcacactcaagatcagcagagtggaggctgaggatgttggagtttattactgctttcaaggttcacatgttcctttcacttttggccaagggaccaagctggagatcaaa

SEQ ID NO: 66 - protein, 112 aa, Artificial Sequence
  Synthetic Construct
DVLMTQSPLSLPVTLGQPASISCRSSQSIVHSNGNTYLEWYQQRPGQSPRLLIYKVSNRFSGVPDRFSGSGSGTDFTLKISRVEAEDVGVYYCFQGSHVPFTFGQGTKLEIK

SEQ ID NO: 67 - DNA, 336 bp, Artificial Sequence
  Synthetic Construct
gatgttgtgatgacccaatctccactctccctgcctgtcacccttggacagccggcctccatctcttgcagatctagtcagagcattgtacatagtaatggaaacacctatttagaatggtaccagcagaggccaggccagtctccaaggctgctgatctacaaagtttccaaccgattttctggggtcccagacaggttcagtggcagtggatcagggacagatttcacactcaagatcagcagagtggaggctgaggatgttggagtttattactgctttcaaggttcacatgttcctttcacttttggccaagggaccaagctggagatcaaa

SEQ ID NO: 68 - protein, 112 aa, Artificial Sequence
  Synthetic Construct
DVVMTQSPLSLPVTLGQPASISCRSSQSIVHSNGNTYLEWYQQRPGQSPRLLIYKVSNRFSGVPDRFSGSGSGTDFTLKISRVEAEDVGVYYCFQGSHVPFTFGQGTKLEIK

SEQ ID NO: 69 - DNA, 984 bp, Artificial Sequence
  Synthetic Construct
gcttccaccaagggcccatccgtcttccccctggcgccctgctccaggagcacctccgagagcacagccgccctgggctgcctggtcaaggactacttccccgaaccggtgacggtgtcgtggaactcaggcgccctgaccagcggcgtgcacaccttcccggctgtcctacagtcctcaggactctactccctcagcagcgtggtgaccgtgccctccagcagcttgggcacgaagacctacacctgcaatgtagatcacaagcccagcaacaccaaggtggacaagagagttgagtccaaatatggtcccccatgcccaccatgcccagcacctgagttcctggggggaccatcagtcttcctgttccccccaaaacccaaggacactctcatgatctcccggacccctgaggtcacgtgcgtggtggtggacgtgagccaggaagaccccgaggtccagttcaactggtacgtggatggcgtggaggtgcataatgccaagacaaagccgcgggaggagcagttcaacagcacgtaccgtgtggtcagcgtcctcaccgtcctgcaccaggactggctgaacggcaaggagtacaagtgcaaggtctccaacaaaggcctcccgtcctccatcgagaaaaccatctccaaagccaaagggcagccccgagagccacaggtgtacaccctgcccccatcccaggaggagatgaccaagaaccaggtcagcctgacctgcctggtcaaaggcttctaccccagcgacatcgccgtggagtgggagagcaatgggcagccggagaacaactacaagaccacgcctcccgtgctggactccgacggctccttcttcctctacagcaggctaaccgtggacaagagcaggtggcaggaggggaatgtcttctcatgctccgtgatgcatgaggctctgcacaaccactacacacagaagagcctctccctgtctctgggtaaatga

SEQ ID NO: 70 - protein, 327 aa, Artificial Sequence
  Synthetic Construct
ASTKGPSVFPLAPCSRSTSESTAALGCLVKDYFPEPVTVSWNSGALTSGVHTFPAVLQSSGLYSLSSVVTVPSSSLGTKTYTCNVDHKPSNTKVDKRVESKYGPPCPPCPAPEFLGGPSVFLFPPKPKDTLMISRTPEVTCVVVDVSQEDPEVQFNWYVDGVEVHNAKTKPREEQFNSTYRVVSVLTVLHQDWLNGKEYKCKVSNKGLPSSIEKTISKAKGQPREPQVYTLPPSQEEMTKNQVSLTCLVKGFYPSDIAVEWESNGQPENNYKTTPPVLDSDGSFFLYSRLTVDKSRWQEGNVFSCSVMHEALHNHYTQKSLSLSLGK

SEQ ID NO: 71 - DNA, 324 bp, Artificial Sequence
  Synthetic Construct
cgaactgtggctgcaccatctgtcttcatcttcccgccatctgatgagcagttgaaatctggaactgcctctgttgtgtgcctgctgaataacttctatcccagagaggccaaagtacagtggaaggtggataacgccctccaatcgggtaactcccaggagagtgtcacagagcaggacagcaaggacagcacctacagcctcagcagcaccctgacgctgagcaaagcagactacgagaaacacaaagtctacgcctgcgaagtcacccatcagggcctgagctcgcccgtcacaaagagcttcaacaggggagagtgttag

SEQ ID NO: 72 - protein, 107 aa, Artificial Sequence [sequence omitted]

SEQ ID NO: 73 - protein, 42 aa, Homo Sapiens [sequence omitted]

SEQ ID NO: 74 - protein, 8 aa, Mus Musculus
GYSFTSYW

SEQ ID NO: 75 - protein, 9 aa, Mus Musculus
VHPGRGVST

SEQ ID NO: 76 - protein, 13 aa, Mus Musculus
SRSHGNTYWFFDV

SEQ ID NO: 77 - protein, 11 aa, Mus Musculus
QSIVHSNGNTY

SEQ ID NO: 78 - protein, 3 aa, Mus Musculus
KVS

SEQ ID NO: 79 - protein, 9 aa, Mus Musculus
FQGSHVPFT

SEQ ID NO: 80 - protein, 16 aa, Mus Musculus
ARDYYGSNSYTSGFAY

SEQ ID NO: 81 - protein, 11 aa, Mus Musculus
QSIVHSNGNTY

SEQ ID NO: 82 - protein, 3 aa, Mus Musculus
KVS

SEQ ID NO: 83 - protein, 9 aa, Mus Musculus
FQGSHVPLT

SEQ ID NO: 84 - DNA, 426 bp, Mus Musculus
atgaacttcgggctcagcttgattttccttgtccttgttttaaaaggtgtccagtgtgaagtgcagctggtggagtctgggggaggcttagtgaagcctggagggtccctgaaactctcctgtgcagcctctggattcactttcagtgactattacatgtattgggttcgccagactccggaaaagaggctggagtgggtcgcaaccattagtgatggtggtagttacacctcctatccagacagtgtgaaggggcgattcaccatctccagagacagtgccaagaacaacctgtacctgcaaatgagcagtctgaagtctgaggacacagccatgtattactgtgcaagagattactacggtagtaatagttacacctcgggctttgcttactggggccaagggactctggtcactgtctctgca

SEQ ID NO: 85 - protein, 142 aa, Mus Musculus
MNFGLSLIFLVLVLKGVQCEVQLVESGGGLVKPGGSLKLSCAASGFTFSDYYMYWVRQTPEKRLEWVATISDGGSYTSYPDSVKGRFTISRDSAKNNLYLQMSSLKSEDTAMYYCARDYYGSNSYTSGFAYWGQGTLVTVSA

SEQ ID NO: 86 - DNA, 396 bp, Mus Musculus
atggattcacaggcccaggttcttatattgctgctgctatgggtatctggtacctgtggggacattgtgatgtcacagtctccatcctccctggctgtgtcagcaggagagaaggtcactatgagctgcaaatccagtcagagtctgctcaatagtagaacccgaaagaactacttggcttggtaccagcagaaaccagggcagtctcctaaactgctgatctactgggcatccactagggaatctggggtccctgatcgcttcacaggcagtggatctgggacagatttcactctcaccatcagcagtgtgcaggctgaagacctggcagtttattactgcaagcaatcttataatctgtacacgttcggaggggggaccaagctggaaataaaa

SEQ ID NO: 87 - protein, 132 aa, Mus Musculus
MDSQAQVLILLLLWVSGTCGDIVMSQSPSSLAVSAGEKVTMSCKSSQSLLNSRTRKNYLAWYQQKPGQSPKLLIYWASTRESGVPDRFTGSGSGTDFTLTISSVQAEDLAVYYCKQSYNLYTFGGGTKLEIK

SEQ ID NO: 88 - DNA, 393 bp, Mus Musculus
atgaagttgcctgttaggctgttggtgctgatgttctggattcctgcttccagcagtgatgttttgatgacccaaactccactctccctgcctgtcagtcttggagatcaagcctccatctcttgcagatctagtcagagcattgtacatagtaatggaaacacctatttagaatggtacctgcagaaaccaggccagtctccaaagctcctgatctacaaagtttccaaccgattttctggggtcccagacaggttcagtggcagtggatcagggacagatttcacactcaagatcagcagagtggaggctgaggatctgggagtttatttctgctttcaaggttcacatgttcctctcacgttcggtgctgggaccaagctggagctgaaa

SEQ ID NO: 89 - protein, 131 aa, Mus Musculus
MKLPVRLLVLMFWIPASSSDVLMTQTPLSLPVSLGDQASISCRSSQSIVHSNGNTYLEWYLQKPGQSPKLLIYKVSNRFSGVPDRFSGSGSGTDFTLKISRVEAEDLGVYFCFQGSHVPLTFGAGTKLELK

SEQ ID NO: 90 - DNA, 1338 bp, Artificial Sequence
  Synthetic Construct
caggtgcagctgcagcagcctggcgctgagctggtgaagcctggagcctccgtgaagatgtcctgcaaggcctccggctactccttcaccagctactggatcaactgggtgaagcagaggcccggacagggcctggagtggattggagacgtgcaccctggccggggagtgtccacctacaacgccaagttcaagtccaaggccaccctgaccctggacacctccagctccaccgcctacatgcagctgtcctccctgacctccgaggactccgccgtgtactactgcagcaggtcccacggcaacacctactggtttttcgacgtgtggggcgccggaaccacagtgaccgtgtcctccgccaaaacgacacccccatctgtctatccactggcccctggatctgctgcccaaactaactccatggtgaccctgggatgcctggtcaagggctatttccctgagccagtgacagtgacctggaactctggatccctgtccagcggtgtgcacaccttcccagctgtcctggagtctgacctctacactctgagcagctcagtgactgtcccctccagccctcggcccagcgagaccgtcacctgcaacgttgcccacccggccagcagcaccaaggtggacaagaaaattgtgcccagggattgtggttgtaagccttgcatatgtacagtcccagaagtatcatctgtcttcatcttccccccaaagcccaaggatgtgctcaccattactctgactcctaaggtcacgtgtgttgtggtagacatcagcaaggatgatcccgaggtccagttcagctggtttgtagatgatgtggaggtgcacacagctcagacgcaaccccgggaggagcagttcaacagcactttccgctcagtcagtgaacttcccatcatgcaccaggactggctcaatggcaaggagttcaaatgcagggtcaacagtgcagctttccctgcccccatcgagaaaaccatctccaaaaccaaaggcagaccgaaggctccacaggtgtacaccattccacctcccaaggagcagatggccaaggataaagtcagtctgacctgcatgataacagacttcttccctgaagacattactgtggagtggcagtggaatgggcagccagcggagaactacaagaacactcagcccatcatgaacacgaatggctcttacttcgtctacagcaagctcaatgtgcagaagagcaactgggaggcaggaaatactttcacctgctctgtgttacatgagggcctgcacaaccaccatactgagaagagcctctcccactctcctggtaaatgatga

SEQ ID NO: 91 - protein, 444 aa, Artificial Sequence
  Synthetic Construct
QVQLQQPGAELVKPGASVKMSCKASGYSFTSYWINWVKQRPGQGLEWIGDVHPGRGVSTYNAKFKSKATLTLDTSSSTAYMQLSSLTSEDSAVYYCSRSHGNTYWFFDVWGAGTTVTVSSAKTTPPSVYPLAPGSAAQTNSMVTLGCLVKGYFPEPVTVTWNSGSLSSGVHTFPAVLESDLYTLSSSVTVPSSPRPSETVTCNVAHPASSTKVDKKIVPRDCGCKPCICTVPEVSSVFIFPPKPKDVLTITLTPKVTCVVVDISKDDPEVQFSWFVDDVEVHTAQTQPREEQFNSTFRSVSELPIMHQDWLNGKEFKCRVNSAAFPAPIEKTISKTKGRPKAPQVYTIPPPKEQMAKDKVSLTCMITDFFPEDITVEWQWNGQPAENYKNTQPIMNTNGSYFVYSKLNVQKSNWEAGNTFTCSVLHEGLHNHHTEKSLSHSPGK

SEQ ID NO: 92 - DNA, 1356 bp, Artificial Sequence
  Synthetic Construct
caggtgcagctgcagcagcctggcgctgagctggtgaagcctggagcctccgtgaagatgtcctgcaaggcctccggctactccttcaccagctactggatcaactgggtgaagcagaggcccggacagggcctggagtggattggagacgtgcaccctggccggggagtgtccacctacaacgccaagttcaagtccaaggccaccctgaccctggacacctccagctccaccgcctacatgcagctgtcctccctgacctccgaggactccgccgtgtactactgcagcaggtcccacggcaacacctactggtttttcgacgtgtggggcgccggaaccacagtgaccgtgtcctccgccaaaacaacagccccatcggtctatccactggcccctgtgtgtggagatacaactggctcctcggtgactctaggatgcctggtcaagggttatttccctgagccagtgaccttgacctggaactctggatccctgtccagtggtgtgcacaccttcccagctgtcctgcagtctgacctctacaccctcagcagctcagtgactgtaacctcgagcacctggcccagccagtccatcacctgcaatgtggcccacccggcaagcagcaccaaggtggacaagaaaattgagcccagagggcccacaatcaagccctgtcctccatgcaaatgcccagcacctaacctcttgggtggaccatccgtcttcatcttccctccaaagatcaaggatgtactcatgatctccctgagccccatagtcacatgtgtggtggtggatgtgagcgaggatgacccagatgtccagatcagctggtttgtgaacaacgtggaagtacacacagctcagacacaaacccatagagaggattacaacagtactctccgggtggtcagtgccctccccatccagcaccaggactggatgagtggcaaggagttcaaatgcaaggtcaacaacaaagacctcccagcgcccatcgagagaaccatctcaaaacccaaagggtcagtaagagctccacaggtatatgtcttgcctccaccagaagaagagatgactaagaaacaggtcactctgacctgcatggtcacagacttcatgcctgaagacatttacgtggagtggaccaacaacgggaaaacagagctaaactacaagaacactgaaccagtcctggactctgatggttcttacttcatgtacagcaagctgagagtggaaaagaagaactgggtggaaagaaatagctactcctgttcagtggtccacgagggtctgcacaatcaccacacgactaagagcttctcccggactccgggtaaatgatga

SEQ ID NO: 93 - protein, 450 aa, Artificial Sequence
  Synthetic Construct
QVQLQQPGAELVKPGASVKMSCKASGYSFTSYWINWVKQRPGQGLEWIGDVHPGRGVSTYNAKFKSKATLTLDTSSSTAYMQLSSLTSEDSAVYYCSRSHGNTYWFFDVWGAGTTVTVSSAKTTAPSVYPLAPVCGDTTGSSVTLGCLVKGYFPEPVTLTWNSGSLSSGVHTFPAVLQSDLYTLSSSVTVTSSTWPSQSITCNVAHPASSTKVDKKIEPRGPTIKPCPPCKCPAPNLLGGPSVFIFPPKIKDVLMISLSPIVTCVVVDVSEDDPDVQISWFVNNVEVHTAQTQTHREDYNSTLRVVSALPIQHQDWMSGKEFKCKVNNKDLPAPIERTISKPKGSVRAPQVYVLPPPEEEMTKKQVTLTCMVTDFMPEDIYVEWTNNGKTELNYKNTEPVLDSDGSYFMYSKLRVEKKNWVERNSYSCSVVHEGLHNHHTTKSFSRTPGK

SEQ ID NO: 94 - DNA, 720 bp, Artificial Sequence
  Synthetic Construct
atgaaactgcccgtgaggctgctggtgctcatgttctggatccctgcctccagctccgatgtgctgatgacccagacccctctgtccctgcctgtgtccctgggcgatcaggccagcatctcctgcaggtcctcccagtccatcgtgcactccaacggcaacacctacctggagtggtacctgcagaagcccggccagtcccccaagctgctgatctacaaggtgtccaaccggttctccggcgtgcccgataggttctccggatccggctccggcaccgactttaccctgaagatctccagggtggaggccgaggacctgggcgtgtactactgctttcagggctcccacgtgcccttcaccttcggctccggcaccaagctggagatcaagcgggctgatgctgcaccaactgtatccatcttcccaccatccagtgagcagttaacatctggaggtgcctcagtcgtgtgcttcttgaacaacttctaccccaaagacatcaatgtcaagtggaagattgatggcagtgaacgacaaaatggcgtcctgaacagttggactgatcaggacagcaaagacagcacctacagcatgagcagcaccctcacgttgaccaaggacgagtatgaacgacataacagctatacctgtgaggccactcacaagacatcaacttcacccattgtcaagagcttcaacaggaatgagtgttgatga

SEQ ID NO: 95 - protein, 219 aa, Artificial Sequence
  Synthetic Construct
DVLMTQTPLSLPVSLGDQASISCRSSQSIVHSNGNTYLEWYLQKPGQSPKLLIYKVSNRFSGVPDRFSGSGSGTDFTLKISRVEAEDLGVYYCFQGSHVPFTFGSGTKLEIKRADAAPTVSIFPPSSEQLTSGGASVVCFLNNFYPKDINVKWKIDGSERQNGVLNSWTDQDSKDSTYSMSSTLTLTKDEYERHNSYTCEATHKTSTSPIVKSFNRNEC

SEQ ID NO: 96 - DNA, 438 bp, Artificial Sequence
  Synthetic Construct
atgggatggagctgtatcatcctctttttggtagcaacagctacaggtgtccactcccaggtccaactgcagcagcctggggctgagcttgtgaagcctggggcttcagtgaaaatgtcctgcaaggcttctggctacagcttcaccagctactggataaactgggtgaagcagaggcctggacaaggccttgagtggattggagatgttcatcctggtagaggtgtttctacctacaatgcgaagttcaagagcaaggccacactgactctagacacgtcctccagcacagcctacatgcagctcagcagcctgacatctgaggactctgcggtctattattgttcaagatcccacggtaatacctactggttcttcgatgtctggggcgcagggaccacggtcaccgtctcctcagctacaacaacagccccatct

SEQ ID NO: 97 - protein, 146 aa, Artificial Sequence
  Synthetic Construct
MGWSCIILFLVATATGVHSQVQLQQPGAELVKPGASVKMSCKASGYSFTSYWINWVKQRPGQGLEWIGDVHPGRGVSTYNAKFKSKATLTLDTSSSTAYMQLSSLTSEDSAVYYCSRSHGNTYWFFDVWGAGTTVTVSSATTTAPS

SEQ ID NO: 98 - DNA, 405 bp, Artificial Sequence
  Synthetic Construct
atgaagttgcctgttaggctgttggtgctgatgttctggattcctgcttccagcagtgatgttttgatgacccaaactccactctccctgcctgtcagtcttggagatcaagcctccatctcttgcagatctagtcagagcattgtacatagtaatggaaacacctatttagaatggtacctgcagaaaccaggccagtctccaaagctcctgatctacaaagtttccaaccgattttctggggtcccagacaggttcagtggcagtggatcagggacagatttcacactcaagatcagcagagtggaggctgaggatctgggagtttattactgctttcaaggttcacatgttccattcacgttcggctcggggacaaagttggaaataaaacgggctgatgct

SEQ ID NO: 99 - protein, 135 aa, Artificial Sequence
  Synthetic Construct
MKLPVRLLVLMFWIPASSSDVLMTQTPLSLPVSLGDQASISCRSSQSIVHSNGNTYLEWYLQKPGQSPKLLIYKVSNRFSGVPDRFSGSGSGTDFTLKISRVEAEDLGVYYCFQGSHVPFTFGSGTKLEIKRADA